European Patent Specification EP 3 967 771 B1, published October 4, 2023. Title: PROBES FOR IMPROVED MELT DISCRIMINATION AND MULTIPLEXING IN NUCLEIC ACIDS ASSAYS. Applicant: LUMINEX CORPORATION. The sequence listing filed with the application follows.

SEQUENCE LISTING (31 sequences)

SEQ ID NO: 1 - DNA, 29 bp, Artificial Sequence
  Synthetic probe
atatcagtcattgcccaaaccgcaatgac

SEQ ID NO: 2 - DNA, 34 bp, Artificial Sequence
  Synthetic probe
atatcagtcattgcccaaaaaaaaccgcaatgac

SEQ ID NO: 3 - DNA, 27 bp, Artificial Sequence
  Synthetic probe
atatcagtcttgcccaaaccgcaagac

SEQ ID NO: 4 - DNA, 32 bp, Artificial Sequence
  Synthetic probe
atatcagtcttgcccaaaaaaaaccgcaagac

SEQ ID NO: 5 - DNA, 31 bp, Artificial Sequence
  Synthetic probe
atatcagtcaattgcccaaaccgcaattgac

SEQ ID NO: 6 - DNA, 36 bp, Artificial Sequence
  Synthetic probe
atatcagtcaattgcccaaaaaaaaccgcaattgac

SEQ ID NO: 7 - DNA, 29 bp, Artificial Sequence
  Synthetic probe
atatcagtcaagtgccaaacccacttgac

SEQ ID NO: 8 - DNA, 34 bp, Artificial Sequence
  Synthetic probe
atatcagtcaagtgccaaaaaaaacccacttgac

SEQ ID NO: 9 - DNA, 25 bp, Artificial Sequence
  Synthetic probe
atatcaggtcagccaaaccctgacc

SEQ ID NO: 10 - DNA, 25 bp, Artificial Sequence
  Synthetic probe
atatcagtctgcccaaaccgcagac

SEQ ID NO: 11 - DNA, 23 bp, Artificial Sequence
  Synthetic probe
atatcagtcgcccaaaccgcgac

SEQ ID NO: 12 - DNA, 66 bp, Artificial Sequence
  Synthetic probe
  modified_base (42)..(42): ribocytosine
atatcagtcattgcccaaaaaaaaaaaaaaaaccgcaatgaccatgagacagtatagtagcgctga

SEQ ID NO: 13 - DNA, 58 bp, Artificial Sequence
  Synthetic probe
  modified_base (35)..(35): ribocytosine
atatcagtcattgcccaaaaaaaaccgcaatgaccatgagacagtatagtagcgctga

SEQ ID NO: 14 - DNA, 60 bp, Artificial Sequence
  Synthetic probe
  modified_base (37)..(37): ribocytosine
atatcagtcatgtgcccaaaaaaaaccgcacatgaccatgagacagtatagtagcgctga

SEQ ID NO: 15 - DNA, 60 bp, Artificial Sequence
  Synthetic probe
  modified_base (37)..(37): ribocytosine
atatcagtcatttgcccaaaaaaaaccgcaaatgaccatgagacagtatagtagcgctga

SEQ ID NO: 16 - DNA, 60 bp, Artificial Sequence
  Synthetic probe
  modified_base (37)..(37): ribocytosine
atatcagtcaattgcccaaaaaaaaccgcaattgaccatgagacagtatagtagcgctga

SEQ ID NO: 17 - DNA, 58 bp, Artificial Sequence
  Synthetic probe
  modified_base (35)..(35): ribocytosine
atatcagtcattgaccaaaaaaaacctcaatgaccatgagacagtatagtagcgctga

SEQ ID NO: 18 - DNA, 58 bp, Artificial Sequence
  Synthetic probe
  modified_base (35)..(35): ribocytosine
atatcagtcattacccaaaaaaaaccgtaatgaccatgagacagtatagtagcgctga

SEQ ID NO: 19 - DNA, 60 bp, Artificial Sequence
  Synthetic probe
  modified_base (37)..(37): ribocytosine
atatcagtcatgtacccaaaaaaaaccgtacatgaccatgagacagtatagtagcgctga

SEQ ID NO: 20 - DNA, 62 bp, Artificial Sequence
  Synthetic probe
  modified_base (39)..(39): ribocytosine
atatcagtcattgtacccaaaaaaaaccgtacaatgaccatgagacagtatagtagcgctga

SEQ ID NO: 21 - DNA, 70 bp, Artificial Sequence
  Synthetic probe
  modified_base (47)..(47): ribocytosine
atatcagtcaatgtgcccaaaaaaaaaaaaaaaaccgcacattgaccatgagacagtatagtagcgctga

SEQ ID NO: 22 - DNA, 23 bp, Artificial Sequence
  Synthetic primer
gaagcatttgaaatagcagaagg

SEQ ID NO: 23 - DNA, 23 bp, Artificial Sequence
  Synthetic primer
cacagagcgttcctagttttact

SEQ ID NO: 24 - DNA, 21 bp, Artificial Sequence
  Synthetic probe
atatcagtcatttgcccaaaa

SEQ ID NO: 25 - DNA, 38 bp, Artificial Sequence
  Synthetic probe
  modified_base (15)..(15): ribocytosine
aaaccgcaaatgaccatgagacagtatagtagcgctga

SEQ ID NO: 26 - DNA, 24 bp, Artificial Sequence
  Synthetic probe
caaaaaaaagtcatgttaccaaaa

SEQ ID NO: 27 - DNA, 34 bp, Artificial Sequence
  Synthetic probe
  modified_base (15)..(15): ribocytosine
aaacctaacatgaccatgagacagtatagtagcg

SEQ ID NO: 28 - DNA, 32 bp, Artificial Sequence
  Synthetic probe
catatcatcatcatctcattttaggcccaaaa

SEQ ID NO: 29 - DNA, 33 bp, Artificial Sequence
  Synthetic probe
  modified_base (15)..(15): ribocytosine
aaaccgcctaaaatccccttagtcagaggtgac

SEQ ID NO: 30 - DNA, 36 bp, Artificial Sequence
  Synthetic probe
ctccatcctcctcctcctctctcttcgagaccaaaa

SEQ ID NO: 31 - DNA, 26 bp, Artificial Sequence
  Synthetic probe
  modified_base (14)..(14): ribocytosine
aaacctctcgaagcgtcctgtccggc